European Patent Application EP 4 461 749 A1, published November 13, 2024. Title: PHARMACEUTICAL COMPOSITION COMPRISING ANTI-FXI/FXIA ANTIBODY AND USE THEREOF. Applicant: Shanghai MabGen Biotech Ltd. The sequence listing filed with the application follows.

SEQUENCE LISTING (24 sequences)

SEQ ID NO: 1 - protein, 607 aa, Homo sapiens
ECVTQLLKDTCFEGGDITTVFTPSAKYCQVVCTYHPRCLLFTFTAESPSEDPTRWFTCVLKDSVTETLPRVNRTAAISGYSFKQCSHQISACNKDIYVDLDMKGINYNSSVAKSAQECQERCTDDVHCHFFTYATRQFPSLEHRNICLLKHTQTGTPTRITKLDKVVSGFSLKSCALSNLACIRDIFPNTVFADSNIDSVMAPDAFVCGRICTHHPGCLFFTFFSQEWPKESQRNLCLLKTSESGLPSTRIKKSKALSGFSLQSCRHSIPVFCHSSFYHDTDFLGEELDIVAAKSHEACQKLCTNAVRCQFFTYTPAQASCNEGKGKCYLKLSSNGSPTKILHGRGGISGYTLRLCKMDNECTTKIKPRIVGGTASVRGEWPWQVTLHTTSPTQRHLCGGSIIGNQWILTAAHCFYGVESPKILRVYSGILNQSEIKEDTSFFGVQEIIIHDQYKMAESGYDIALLKLETTVNYTDSQRPICLPSKGDRNVIYTDCWVTGWGYRKLRDKIQNTLQKAKIPLVTNEECQKRYRGHKITHKMICAGYREGGKDACKGDSGGPLSCKHNEVWHLVGITSWGEGCAQRERPGVYTNVVEYVDWILEKTQAV

SEQ ID NO: 2 - protein, 18 aa, synthetic construct
  source 1..18: note; note (original language) = FXIa-specific polypeptide
CFYGVESPKILRVYSGIL

SEQ ID NO: 3 - protein, 21 aa, synthetic construct
  source 1..21: note; note (original language) = FXIa-specific polypeptide
CGYRKLRDKIQNTLQKAKIPL

SEQ ID NO: 4 - protein, 21 aa, synthetic construct
  source 1..21: note; note (original language) = FXIa-specific polypeptide
CGVQEIIIHDQYKMAESGYDI

SEQ ID NO: 5 - protein, 117 aa, synthetic construct
  source 1..117: note = 3807-VH
EVQLQQSGAELVRPGTSVKLSCIASGFNIKDDYMHWVKQRPEQGLEWIGWIDPENGDTEYASKFQGKATITADTSANTAYLQFSSLTSEDTAVYYCLYGNFYYFDYWGQGTTLTVSS

SEQ ID NO: 6 - protein, 106 aa, synthetic construct
  source 1..106: note = 3807-VL
QIVLTQSPAIMSASPGEKVTMTCSASSSINYMHWYQQKPGTSPKRWIYDTSKLASGVPARFSGSGSGTSYSLTISSMEAEDAATYYCHQRSFSPLTFGAGTKLELK

SEQ ID NO: 7 - protein, 5 aa, synthetic construct
  source 1..5: note = 3807-HCDR1
DDYMH

SEQ ID NO: 8 - protein, 17 aa, synthetic construct
  source 1..17: note = 3807-HCDR2
WIDPENGDTEYASKFQG

SEQ ID NO: 9 - protein, 8 aa, synthetic construct
  source 1..8: note = 3807-HCDR3
GNFYYFDY

SEQ ID NO: 10 - protein, 10 aa, synthetic construct
  source 1..10: note = 3807-LCDR1
SASSSINYMH

SEQ ID NO: 11 - protein, 7 aa, synthetic construct
  source 1..7: note = 3807-LCDR2
DTSKLAS

SEQ ID NO: 12 - protein, 9 aa, synthetic construct
  source 1..9: note = 3807-LCDR3
HQRSFSPLT

SEQ ID NO: 13 - protein, 117 aa, synthetic construct
  source 1..117: note = 3807VH-CDR graft
QVQLVQSGAEVKKPGSSVKVSCKASGYTFTDDYMHWVRQAPGQGLEWMGWIDPENGDTEYASKFQGRVTITADESTSTAYMELSSLRSEDTAVYYCARGNFYYFDYWGQGTTVTVSS

SEQ ID NO: 14 - protein, 106 aa, synthetic construct
  source 1..106: note = 3807VL-CDR graft
EIVLTQSPATLSLSPGERATLSCSASSSINYMHWYQQKPGQAPRLLIYDTSKLASGIPARFSGSGSGTDFTLTISSLEPEDFAVYYCHQRSFSPLTFGQGTKLEIK

SEQ ID NO: 15 - protein, 117 aa, synthetic construct
  source 1..117: note = 3807-VH1
QVQLVQSGAEVKKPGSSVKVSCKASGFNIKDDYMHWVRQAPGQGLEWMGWIDPENGDTEYASKFQGRVTITADESTSTAYMELSSLRSEDTAVYYCLYGNFYYFDYWGQGTTVTVSS

SEQ ID NO: 16 - protein, 106 aa, synthetic construct
  source 1..106: note = 3807-VL3
EIVLTQSPATLSLSPGERATLSCSASSSINYMHWYQQKPGQAPKRWIYDTSKLASGVPARFSGSGSGTDFTLTISSLEPEDFAVYYCHQRSFSPLTFGQGTKLEIK

SEQ ID NO: 17 - protein, 117 aa, synthetic construct
  source 1..117: note = 3807-VH1(GTFS)
QVQLVQSGAEVKKPGSSVKVSCKASGGTFSDDYMHWVRQAPGQGLEWMGWIDPENGDTEYASKFQGRVTITADESTSTAYMELSSLRSEDTAVYYCLYGNFYYFDYWGQGTTVTVSS

SEQ ID NO: 18 - protein, 98 aa, Homo sapiens
ASTKGPSVFPLAPCSRSTSESTAALGCLVKDYFPEPVTVSWNSGALTSGVHTFPAVLQSSGLYSLSSVVTVPSSSLGTKTYTCNVDHKPSNTKVDKRV

SEQ ID NO: 19 - protein, 229 aa, synthetic construct
  source 1..229: note = IgG4 FcS241P
ESKYGPPCPPCPAPEFLGGPSVFLFPPKPKDTLMISRTPEVTCVVVDVSQEDPEVQFNWYVDGVEVHNAKTKPREEQFNSTYRVVSVLTVLHQDWLNGKEYKCKVSNKGLPSSIEKTISKAKGQPREPQVYTLPPSQEEMTKNQVSLTCLVKGFYPSDIAVEWESNGQPENNYKTTPPVLDSDGSFFLYSRLTVDKSRWQEGNVFSCSVMHEALHNHYTQKSLSLSLGK

SEQ ID NO: 20 - protein, 107 aa, Homo sapiens [sequence omitted]

SEQ ID NO: 21 - protein, 444 aa, synthetic construct
  source 1..444: note = 3882-HC
QVQLVQSGAEVKKPGSSVKVSCKASGGTFSDDYMHWVRQAPGQGLEWMGWIDPENGDTEYASKFQGRVTITADESTSTAYMELSSLRSEDTAVYYCLYGNFYYFDYWGQGTTVTVSSASTKGPSVFPLAPCSRSTSESTAALGCLVKDYFPEPVTVSWNSGALTSGVHTFPAVLQSSGLYSLSSVVTVPSSSLGTKTYTCNVDHKPSNTKVDKRVESKYGPPCPPCPAPEFLGGPSVFLFPPKPKDTLMISRTPEVTCVVVDVSQEDPEVQFNWYVDGVEVHNAKTKPREEQFNSTYRVVSVLTVLHQDWLNGKEYKCKVSNKGLPSSIEKTISKAKGQPREPQVYTLPPSQEEMTKNQVSLTCLVKGFYPSDIAVEWESNGQPENNYKTTPPVLDSDGSFFLYSRLTVDKSRWQEGNVFSCSVMHEALHNHYTQKSLSLSLGK

SEQ ID NO: 22 - protein, 213 aa, synthetic construct
  source 1..213: note = 3882-LC
EIVLTQSPATLSLSPGERATLSCSASSSINYMHWYQQKPGQAPKRWIYDTSKLASGVPARFSGSGSGTDFTLTISSLEPEDFAVYYCHQRSFSPLTFGQGTKLEIKRTVAAPSVFIFPPSDEQLKSGTASVVCLLNNFYPREAKVQWKVDNALQSGNSQESVTEQDSKDSTYSLSSTLTLSKADYEKHKVYACEVTHQGLSSPVTKSFNRGEC

SEQ ID NO: 23 - protein, 449 aa, synthetic construct
  source 1..449: note = BAY1213790
EVQLLESGGGLVQPGGSLRLSCAASGFTFSQYGMDWVRQAPGKGLEWVSGIGPSGGSTVYADSVKGRFTISRDNSKNTLYLQMNSLRAEDTAVYYCTRGGPYYYYGMDVWGQGTTVTVSSASTKGPSVFPLAPSSKSTSGGTAALGCLVKDYFPEPVTVSWNSGALTSGVHTFPAVLQSSGLYSLSSVVTVPSSSLGTQTYICNVNHKPSNTKVDKKVEPKSCDKTHTCPPCPAPELLGGPSVFLFPPKPKDTLMISRTPEVTCVVVDVSHEDPEVKFNWYVDGVEVHNAKTKPREEQYNSTYRVVSVLTVLHQDWLNGKEYKCKVSNKALPAPIEKTISKAKGQPREPQVYTLPPSRDELTKNQVSLTCLVKGFYPSDIAVEWESNGQPENNYKTTPPVLDSDGSFFLYSKLTVDKSRWQQGNVFSCSVMHEALHNHYTQKSLSLSPG

SEQ ID NO: 24 - protein, 214 aa, synthetic construct
  source 1..214: note = BAY1213790
DIQMTQSPSSLSASVGDRVTITCQASQDISNYLNWYQQKPGKAPKLLIYDASNLETGVPSRFSGSGSGTDFTFTISSLQPEDIATYYCQQADSFPVTFGGGTKVEIKRTVAAPSVFIFPPSDEQLKSGTASVVCLLNNFYPREAKVQWKVDNALQSGNSQESVTEQDSKDSTYSLSSTLTLSKADYEKHKVYACEVTHQGLSSPVTKSFNRGEC